European Patent Specification EP 3 625 259 B1, published April 17, 2024. Title: Anti SIRPalpha antibodies with a LALA mutation. Applicant: Synthon Biopharmaceuticals B.V. VERHEIJDEN Gijsbertus Franciscus Maria ROUWENDAL Gerard Johan Adolph ARENDS Roland Jan BERG, VAN DEN Timo Kars MATLUNG Hanke Lottie SZILAGYI Katarina. The sequence listing filed with the application follows.

SEQUENCE LISTING (29 sequences)

SEQ ID NO: 1 - protein, 117 aa, Artificial Sequence
  SEQ ID NO:1 (HC VR 1)
QSVEESGGRLVTPGTPLTLTCTVSGIDLSSYAMSWVRQAPGKGLEWIGIISSGGITYYASWAKGRFTISKTSTTVDLKIPSPTTEDTATYFCARSLWAASNYYMALWGPGTLVTVSS

SEQ ID NO: 2 - protein, 111 aa, Artificial Sequence
  SEQ ID NO:2 (LC VR 1)
AIKMTQTPASVSAAVGGTVSINCQASEDIESYLAWYQQKPGQPPKLLIYRASTLASGVSSRFKGSGSGTQFTLTISDLESADAATYYCLGDYYSSSGDTGAFGGGTEVVVK

SEQ ID NO: 3 - protein, 116 aa, Artificial Sequence
  SEQ ID NO:3 (HC VR 2)
QSVEESGGRLVTPGTPLTLTCTVSGFSLSNYAMHWVRQAPGKGLEWIGIIYTGGATSYATWAKGQFTISKTSTTVDLKITSPTTEDTATYFCARGDRDGYAYFNIWGPGTLVTVSL

SEQ ID NO: 4 - protein, 110 aa, Artificial Sequence
  SEQ ID NO:4 (LC VR 2)
QIVMTQTPFSVSAVVGGTVTIKCQASHNIGSWLAWYQQKPGQRPKLLIYDASTLASGVSSRFKGSGSGTEFTLTISGVESADAATYYCQQGYGISYVHNVFGGGTEVVVK

SEQ ID NO: 5 - protein, 116 aa, Artificial Sequence
  SEQ ID NO:5 (HC VR 3)
QSVEESGGRLVTPGTPLTLACTVSGFSLISYYISWVRQAPEKGLEYIGIINIGGGASYASWAKGRFTISKTSTTVDLKITSPTPEDTATYFCAMSYGMDTGAFNIWGPGTLVTVSL

SEQ ID NO: 6 - protein, 110 aa, Artificial Sequence
  SEQ ID NO:6 (LC VR 3)
AQVLTQTPASVSAAVGGTVTISCQSSESVYKNNFLSWYQQKPGKPPKLLIYGASTLASGVPSRFKGSGSGTQFTLTISDLESDDAATYFCQGGYRTDIYPFGGGTEVVVK

SEQ ID NO: 7 - protein, 116 aa, Artificial Sequence
  SEQ ID NO:7 (HC VR 4)
QSVEESGGRLGTPGTPLTLTCTVSGFSLSSYVMGWFRQAPGKGLEYIGIISSSGSPYYASWVNGRFTISKTSTTMDLKMNSPTTEDTATYFCARVGPLGVDYFNIWGPGTLVTVSL

SEQ ID NO: 8 - protein, 109 aa, Artificial Sequence
  SEQ ID NO:8 (LC VR 4)
DIVMTQTPSSVEAAVGGTVTIKCQAGQSINSYLAWYQQKPGQRPKLLIYYASTLESGVPSRFKGSGSGTDYTLTISDLESADAATYYCQSWHYISRSYAFGGGTEVVVK

SEQ ID NO: 9 - protein, 116 aa, Artificial Sequence
  SEQ ID NO:9 (HC VR 5)
QSVEESGGRLVTPGTPLTLTCTVSGFSLSSYVMGWFRQAAGKGLEYIGYINADGSPYYATWVNGRFTISKTPTTMDLKINSPTTEDTATYFCARVGPLGVDYFNIWGPGTLVTVSL

SEQ ID NO: 10 - protein, 109 aa, Artificial Sequence
  SEQ ID NO:10 (LC VR 5)
DIVMTQTPASVEAAVGGTVTIKCQASQSINRYLTWYQQKPGQRPKLLIYYASTLESGVPSRFEGSGSGTDYTLTISDLESADAATYYCQSYYYISRTYAFGGGTEVVVK

SEQ ID NO: 11 - protein, 116 aa, Artificial Sequence
  SEQ ID NO:11 (HC VR 6)
QSVEESGGRLVTPGTPLTLTCTVSGIDLSSYTMTWVRQAPGKGLEWIGIIYAGGSTAYASWAKGRFTISKTSTTVDLKITSPTTEDTATYFCARSSSDGYDYFNIWGPGTLVTVSL

SEQ ID NO: 12 - protein, 111 aa, Artificial Sequence
  SEQ ID NO:12 (LC VR 6)
GVVMTQTPSSVSAAVGGTVTINCQASQSIGSWLAWYQQKPGQPPKLLIYQASKLASGVPSRFSGRGSGTHFTLTISDVQSDDAATYYCQQTVTAASNVDNAFGGGTEVVVK

SEQ ID NO: 13 - protein, 115 aa, Artificial Sequence
  SEQ ID NO:13 (HC VR 7)
RSVEESGGRLVTPGTPLTLTCTVSGFSLSSHGISWVRQAPGKGLEYIGTIGTGVITYFASWAKGRFTGSKTSTTVDLKITSPTTEDTATYFCARGSAWNDPFDPWGPGTLVTVSS

SEQ ID NO: 14 - protein, 111 aa, Artificial Sequence
  SEQ ID NO:14 (LC VR 7)
ALVMTQTPASVSAAVGGTVTTKCQASQSVYGNNDLAWYQHKPGQPPKLLIYLASTLATGVPSRFSGSGSGTQFTLTITGVQSDDAATYYCLGGGDDEADNVFGGGTEVVVK

SEQ ID NO: 15 - protein, 116 aa, Artificial Sequence
  SEQ ID NO:15 (HC VR 8)
QSLEESGGRLVTPGTPLTLTCTASGVDLSNYAMGWVRQAPGKGLEWIGIIYAGGSTSYATWAKGRFTISKTSTTMDLKMTSPTTEDTATYFCARHRSDGYDYFHLWGPGTLVTVSL

SEQ ID NO: 16 - protein, 110 aa, Artificial Sequence
  SEQ ID NO:16 (LC VR 8)
AIDMTQTPASVSEPVGGTVTIKCQASQSISSWLAWYQQKPGQRPKLLIYDASKLASGVPSRFSGSGSGTEFTLTISGVQSDDAAAYYCQQGYAVSYVENIFGGGTEVVVK

SEQ ID NO: 17 - protein, 117 aa, Artificial Sequence
  SEQ ID NO:17 (HC VR 9)
QSMEESGGRLVTPGTPLTLTCTASGFSLSNYGVSWVRQAPGKGLEWIGIIYGGSDITAYASWAKGRFTISKTSTTVDLTITSPTTEDTATYFCAKSYTNGMDYYNIWGPGTLVTVSL

SEQ ID NO: 18 - protein, 108 aa, Artificial Sequence
  SEQ ID NO:18 (LC VR 9)
AFDLTQTPSSVEAPVGGTVIIKCQASQSISSYLAWYQQKPGQPPKLLIYSASTLASGVSSRFKGSGSETQFPLTISDLESADAATYYCQSYYGSRSNVFGGGTEVVVK

SEQ ID NO: 19 - protein, 129 aa, Artificial Sequence
  SEQ ID NO:19 (HC VR 29AM4-5))
EVQLVESGGGLVQPGGSLRLSCAASGFNISYYFIHWVRQAPGKGLEWVASVYSSFGYTYYADSVKGRFTISADTSKNTAYLQMNSLRAEDTAVYYCARFTFPGLFDGFFGAYLGSLDYWGQGTLVTVSS

SEQ ID NO: 20 - protein, 110 aa, Artificial Sequence
  SEQ ID NO:20 (LC VR 29AM4-5)
DIQMTQSPSSLSASVGDRVTITCRASQSVSSAVAWYQQKPGKAPKLLIYSASSLYSGVPSRFSGSRSGTDFTLTISSLQPEDFATYYCQQAVNWVGALVTFGQGTKVEIK

SEQ ID NO: 21 - protein, 121 aa, Artificial Sequence
  SEQ ID NO:21 (HC VR 12C4)
EVKLEESGGGLMQPGGSMKLSCVASGFTFSNYWMNWVRQSPEKGLEWVAEIRLKSNNYATHYAESVKGRFTISRDDSKSSVYLQMNNLRAEDTGIYYCIRDYDYDAYFDYWGQGTTLTVSS

SEQ ID NO: 22 - protein, 111 aa, Artificial Sequence
  SEQ ID NO:22 (LC VR 12C4)
DIVLTQSPASLAVSLGQRATISCRASKSVSTSGYNYMYWYQQKPGQPPKLLIYLASNLESGVPARFSGSGSGTDFTLNIHPVEEEDAATYYCQHSGELPYTFGGGTKLEIK

SEQ ID NO: 23 - protein, 113 aa, Artificial Sequence
  SEQ ID NO:23 (HC KWAR23 )
EVQLQQSGAELVKPGASVKLSCTASGFNIKDYYIHWVQQRTEQGLEWIGRIDPEDGETKYAPKFQDKATITADTSSNTAYLHLSSLTSEDTAVYYCARWGAYWGQGTLVTVSS

SEQ ID NO: 24 - protein, 108 aa, Artificial Sequence
  SEQ ID NO:24 (LC VR KWAR23)
QIVLTQSPAIMSASPGEKVTLTCSASSSVSSSYLYWYQQKPGSSPKLWIYSTSNLASGVPARFSGSGSGTSYSLTISSMEAEDAASYFCHQWSSYPRTFGAGTKLELK

SEQ ID NO: 25 - protein, 330 aa, Artificial Sequence [sequence omitted]

SEQ ID NO: 26 - protein, 107 aa, Artificial Sequence [sequence omitted]

SEQ ID NO: 27 - protein, 330 aa, Artificial Sequence
  SEQ ID NO 27: (human IgG1 antibody HC constant region LALA mutant (mutations underlined)
ASTKGPSVFPLAPSSKSTSGGTAALGCLVKDYFPEPVTVSWNSGALTSGVHTFPAVLQSSGLYSLSSVVTVPSSSLGTQTYICNVNHKPSNTKVDKKVEPKSCDKTHTCPPCPAPEAAGGPSVFLFPPKPKDTLMISRTPEVTCVVVDVSHEDPEVKFNWYVDGVEVHNAKTKPREEQYNSTYRVVSVLTVLHQDWLNGKEYKCKVSNKALPAPIEKTISKAKGQPREPQVYTLPPSRDELTKNQVSLTCLVKGFYPSDIAVEWESNGQPENNYKTTPPVLDSDGSFFLYSKLTVDKSRWQQGNVFSCSVMHEALHNHYTQKSLSLSPGK

SEQ ID NO: 28 - protein, 19 aa, Artificial Sequence
  SEQ ID NO:28 (leader sequence antibodies 1-9)
MGWSCIILFLVATATGVHS

SEQ ID NO: 29 - protein, 21 aa, Artificial Sequence
  SEQ ID NO:29 (HAVT20 leader sequence)
MACPGFLWALVISTCLEFSMA